European Patent Application EP 4 130 025 A1, published February 8, 2023. Title: A COMPOSITION FOR TREATING CANCER COMPRISING VGLL1 PEPTIDE. Applicant: Onecuregen Co., Ltd. The sequence listing filed with the application follows.

SEQUENCE LISTING (31 sequences)

SEQ ID NO: 1 - protein, 258 aa, Homo sapiens
  PEPTIDE (1)..(258): VGLL1
MEEMKKTAIRLPKGKQKPIKTEWNSRCVLFTYFQGDISSVVDEHFSRALSNIKSPQELTPSSQSEGVMLKNDDSMSPNQWRYSSPWTKPQPEVPVTNRAANCNLHVPGPMAVNQFSPSLARRASVRPGELWHFSSLAGTSSLEPGYSHPFPARHLVPEPQPDGKREPLLSLLQQDRCLARPQESAARENGNPGQIAGSTGLLFNLPPGSVHYKKLYVSRGSASTSLPNETLSELETPGKYSLTPPNHWGHPHRYLQHL

SEQ ID NO: 2 - protein, 15 aa, Artificial Sequence
  77-91_VGLL1
PNQWRYSSPWTKPQP

SEQ ID NO: 3 - protein, 13 aa, Artificial Sequence
  78-90_VGLL1
NQWRYSSPWTKPQ

SEQ ID NO: 4 - protein, 11 aa, Artificial Sequence
  79-89_VGLL1
QWRYSSPWTKP

SEQ ID NO: 5 - protein, 9 aa, Artificial Sequence
  80-88_VGLL1
WRYSSPWTK

SEQ ID NO: 6 - protein, 8 aa, Artificial Sequence
  80-87_VGLL1
WRYSSPWT

SEQ ID NO: 7 - protein, 7 aa, Artificial Sequence
  80-86_VGLL1
WRYSSPW

SEQ ID NO: 8 - protein, 7 aa, Artificial Sequence
  81-87_VGLL1
RYSSPWT

SEQ ID NO: 9 - protein, 7 aa, Artificial Sequence
  82-88_VGLL1
YSSPWTK

SEQ ID NO: 10 - protein, 15 aa, Artificial Sequence
  P85A variant_VGLL1
PNQWRYSSAWTKPQP

SEQ ID NO: 11 - protein, 15 aa, Artificial Sequence
  T87A variant_VGLL1
PNQWRYSSPWAKPQP

SEQ ID NO: 12 - protein, 11 aa, Artificial Sequence
  HIV-1 Tat
YGRKKRRQRRR

SEQ ID NO: 13 - protein, 16 aa, Artificial Sequence
  Penetratin
RQIKIWFQNRRMKWKK

SEQ ID NO: 14 - protein, 34 aa, Artificial Sequence
  HSV VP22
DAATATRGRSAASRPTERPRAPARSASRPRRPVE

SEQ ID NO: 15 - protein, 14 aa, Artificial Sequence
  MTS
AAVALLPAVLLAAP

SEQ ID NO: 16 - protein, 27 aa, Artificial Sequence
  Transportan
GWTLNSAGYLLGKINLKALAALAKKIL

SEQ ID NO: 17 - protein, 21 aa, Artificial Sequence
  PEP-1
KETWWETWWTEWSQPKKKRKV

SEQ ID NO: 18 - protein, 7 aa, Artificial Sequence
  Poly arginine
RRRRRRR

SEQ ID NO: 19 - protein, 12 aa, Artificial Sequence
  PTD-5
RRQRRTSKLMKR

SEQ ID NO: 20 - DNA, 20 bp, Artificial Sequence
  MMP9 Forward Primer
tctatggtcctcgccctgaa

SEQ ID NO: 21 - DNA, 20 bp, Artificial Sequence
  MMP9 Reverse Primer
catcgtccaccggactcaaa

SEQ ID NO: 22 - RNA, 23 nt, Artificial Sequence
  siMMP9 (22,23-dTdT)
ccacaacaucaccuauuggautt

SEQ ID NO: 23 - RNA, 21 nt, Artificial Sequence
  siSC (20,21-dTdT)
ccuacgccaccaauuucgutt

SEQ ID NO: 24 - RNA, 25 nt, Artificial Sequence
  siVGLL1 (24,25-dTdT)
agccuauaaagacggaauggaautt

SEQ ID NO: 25 - RNA, 21 nt, Artificial Sequence
  siTEAD4 (20,21-dTdT)
gacacuacucuuaccgcautt

SEQ ID NO: 26 - RNA, 23 nt, Artificial Sequence
  siYAP (22,23-dTdT)
ccaccaagcuagauaaagaaatt

SEQ ID NO: 27 - protein, 26 aa, Artificial Sequence
  Tat-VGLL1
YGRKKRRQRRRPNQWRYSSPWTKPQP

SEQ ID NO: 28 - protein, 26 aa, Artificial Sequence
  Tat-VGLL1(S84A)
YGRKKRRQRRRPNQWRYSAPWTKPQP

SEQ ID NO: 29 - protein, 18 aa, Artificial Sequence
  Tat-VGLL1(S84-S)
YGRKKRRQRRRYSSPWTK

SEQ ID NO: 30 - protein, 26 aa, Artificial Sequence
  Tat-VGLL1(P85A)
YGRKKRRQRRRPNQWRYSSAWTKPQP

SEQ ID NO: 31 - protein, 26 aa, Artificial Sequence
  Tat-VGLL1(T87A)
YGRKKRRQRRRPNQWRYSSPWAKPQP